European Patent Specification EP 2 533 763 B1, published July 12, 2023. Title: Dermatologische, pharmazeutische Zusammensetzung geeignet für Oligonukleotide. Applicant: Sterna Biologicals GmbH & Co KG. Application DE 10 2010 007 562.0-41. The sequence listing filed with the application follows.

SEQUENCE LISTING (148 sequences)

SEQ ID NO: 1 - DNA, 33 bp, Homo sapiens
  hgd1 DNAzyme against GATA-3mRNA (1)..(33)
tcggtcagaggctagctacaacgatgcgttgct

SEQ ID NO: 2 - DNA, 33 bp, Homo sapiens
  hdg2 DNAzyme against GATA-3mRNA (1)..(33)
ggcgtacgaggctagctacaacgactgctcggt

SEQ ID NO: 3 - DNA, 33 bp, Homo sapiens
  hgd3 DNAzyme against GATA-3mRNA (1)..(33)
ggcggcgtaggctagctacaacgagacctgctc

SEQ ID NO: 4 - DNA, 33 bp, Homo sapiens
  hgd4 DNAzyme against GATA-3mRNA (1)..(33)
ctcgggtcaggctagctacaacgactgggtagc

SEQ ID NO: 5 - DNA, 33 bp, Homo sapiens
  hgd5 DNAzyme against GATA-3mRNA (1)..(33)
tcctctgcaggctagctacaacgacggggtcct

SEQ ID NO: 6 - DNA, 33 bp, Homo sapiens
  hgd6 DNAzyme against GATA-3mRNA (1)..(33)
actctgcaaggctagctacaacgatctgcgagc

SEQ ID NO: 7 - DNA, 33 bp, Homo sapiens
  hgd7 DNAzyme against GATA-3mRNA (1)..(33)
gggcgacgaggctagctacaacgatctgcaatt

SEQ ID NO: 8 - DNA, 33 bp, Homo sapiens
  hgd8 DNAzyme against GATA-3mRNA (1)..(33)
aaggggcgaggctagctacaacgagactctgca

SEQ ID NO: 9 - DNA, 33 bp, Homo sapiens
  hgd9 DNAzyme against GATA-3mRNA (1)..(33)
aaaacgggaggctagctacaacgacaggttgta

SEQ ID NO: 10 - DNA, 33 bp, Homo sapiens
  hgd10 DNAzyme against GATA-3mRNA (1)..(33)
agaataaaaggctagctacaacgagggaccagg

SEQ ID NO: 11 - DNA, 33 bp, Homo sapiens
  hgd11 DNAzyme against GATA-3mRNA (1)..(33)
atggcagaaggctagctacaacgaaaaacggga

SEQ ID NO: 12 - DNA, 33 bp, Homo sapiens
  hgd12 DNAzyme against GATA-3mRNA (1)..(33)
aactgggtaggctagctacaacgaggcagaata

SEQ ID NO: 13 - DNA, 33 bp, Homo sapiens
  hgd13 DNAzyme against GATA-3mRNA (1)..(33)
atccaaaaaggctagctacaacgatgggtatgg

SEQ ID NO: 14 - DNA, 33 bp, Homo sapiens
  hgd14 DNAzyme against GATA-3mRNA (1)..(33)
aggggaagaggctagctacaacgaaaaaatcca

SEQ ID NO: 15 - DNA, 33 bp, Homo sapiens
  hgd15 DNAzyme against GATA-3mRNA (1)..(33)
ttttaaaaaggctagctacaacgatatcttgga

SEQ ID NO: 16 - DNA, 33 bp, Homo sapiens
  hgd16 DNAzyme against GATA-3mRNA (1)..(33)
gtggggggaggctagctacaacgagggaaggct

SEQ ID NO: 17 - DNA, 33 bp, Homo sapiens
  hgd17 DNAzyme against GATA-3mRNA (1)..(33)
gttgaatgaggctagctacaacgattgctttcg

SEQ ID NO: 18 - DNA, 33 bp, Homo sapiens
  hgd18 DNAzyme against GATA-3mRNA (1)..(33)
gtcgttgaaggctagctacaacgagatttgctt

SEQ ID NO: 19 - DNA, 33 bp, Homo sapiens
  hgd19 DNAzyme against GATA-3mRNA (1)..(33)
ggcccggaaggctagctacaacgaccgcgcgcg

SEQ ID NO: 20 - DNA, 33 bp, Homo sapiens
  hgd20 DNAzyme against GATA-3mRNA (1)..(33)
tcacctccaggctagctacaacgaggcctcggc

SEQ ID NO: 21 - DNA, 33 bp, Homo sapiens
  hgd21 DNAzyme against GATA-3mRNA (1)..(33)
ccgccgtcaggctagctacaacgactccatggc

SEQ ID NO: 22 - DNA, 33 bp, Homo sapiens
  hgd22 DNAzyme against GATA-3mRNA (1)..(33)
ggtggctcaggctagctacaacgaccagcgcgg

SEQ ID NO: 23 - DNA, 33 bp, Homo sapiens
  hgd23 DNAzyme against GATA-3mRNA (1)..(33)
cgttgagcaggctagctacaacgaggcggggtg

SEQ ID NO: 24 - DNA, 33 bp, Homo sapiens
  hgd24 DNAzyme against GATA-3mRNA (1)..(33)
ccgcgtccaggctagctacaacgagtaggagtg

SEQ ID NO: 25 - DNA, 33 bp, Homo sapiens
  hgd25 DNAzyme against GATA-3mRNA (1)..(33)
cagcgggtaggctagctacaacgatgcgccgcg

SEQ ID NO: 26 - DNA, 33 bp, Homo sapiens
  hgd26 DNAzyme against GATA-3mRNA (1)..(33)
gcacatccaggctagctacaacgactcctccgg

SEQ ID NO: 27 - DNA, 33 bp, Homo sapiens
  hgd27 DNAzyme against GATA-3mRNA (1)..(33)
aaaagcacaggctagctacaacgaccacctcct

SEQ ID NO: 28 - DNA, 33 bp, Homo sapiens
  hgd28 DNAzyme against GATA-3mRNA (1)..(33)
taaaaagcaggctagctacaacgaatccacctc

SEQ ID NO: 29 - DNA, 33 bp, Homo sapiens
  hgd29 DNAzyme against GATA-3mRNA (1)..(33)
gaccgtcgaggctagctacaacgagttaaaaag

SEQ ID NO: 30 - DNA, 33 bp, Homo sapiens
  hgd30 DNAzyme against GATA-3mRNA (1)..(33)
ttgccttgaggctagctacaacgacgtcgatgt

SEQ ID NO: 31 - DNA, 33 bp, Homo sapiens
  hgd31 DNAzyme against GATA-3mRNA (1)..(33)
agggcgggaggctagctacaacgagtggttgcc

SEQ ID NO: 32 - DNA, 33 bp, Homo sapiens
  hgd32 DNAzyme against GATA-3mRNA (1)..(33)
tggccctgaggctagctacaacgacgagtttcc

SEQ ID NO: 33 - DNA, 33 bp, Homo sapiens
  hgd33 DNAzyme against GATA-3mRNA (1)..(33)
acctctgcaggctagctacaacgacgtggccct

SEQ ID NO: 34 - DNA, 33 bp, Homo sapiens
  hgd34 DNAzyme against GATA-3mRNA (1)..(33)
cggagggtaggctagctacaacgactctgcacc

SEQ ID NO: 35 - DNA, 33 bp, Homo sapiens
  hgd35 DNAzyme against GATA-3mRNA (1)..(33)
ggcggcacaggctagctacaacgactggctccc

SEQ ID NO: 36 - DNA, 33 bp, Homo sapiens
  hgd36 DNAzyme against GATA-3mRNA (1)..(33)
cgggcggcaggctagctacaacgaacctggctc

SEQ ID NO: 37 - DNA, 33 bp, Homo sapiens
  hgd37 DNAzyme against GATA-3mRNA (1)..(33)
agggatccaggctagctacaacgagaagcagag

SEQ ID NO: 38 - DNA, 33 bp, Homo sapiens
  hgd38 DNAzyme against GATA-3mRNA (1)..(33)
gggtagggaggctagctacaacgaccatgaagc

SEQ ID NO: 39 - DNA, 33 bp, Homo sapiens
  hgd39 DNAzyme against GATA-3mRNA (1)..(33)
gggctgagaggctagctacaacgatccaggggg

SEQ ID NO: 40 - DNA, 33 bp, Homo sapiens
  hgd40 DNAzyme against GATA-3mRNA (1)..(33)
gtggatggaggctagctacaacgagtcttggag

SEQ ID NO: 41 - DNA, 33 bp, Homo sapiens
  hgd 41 DNAzyme against GATA-3mRNA (1)..(33)
cgtggtggaggctagctacaacgaggacgtctt

SEQ ID NO: 42 - DNA, 33 bp, Homo sapiens
  hgd 42 DNAzyme against GATA-3mRNA (1)..(33)
gggggtagaggctagctacaacgaggagagggg

SEQ ID NO: 43 - DNA, 33 bp, Homo sapiens
  hgd 43 DNAzyme against GATA-3mRNA (1)..(33)
ggaggaggaggctagctacaacgagaggccggg

SEQ ID NO: 44 - DNA, 33 bp, Homo sapiens
  hgd44 DNAzyme against GATA-3mRNA (1)..(33)
gccccccgaggctagctacaacgaaaggaggag

SEQ ID NO: 45 - DNA, 33 bp, Homo sapiens
  hgd45 DNAzyme against GATA-3mRNA (1)..(33)
ccggggagaggctagctacaacgagtccttcgg

SEQ ID NO: 46 - DNA, 33 bp, Homo sapiens
  hgd46 DNAzyme against GATA-3mRNA (1)..(33)
ggacagcgaggctagctacaacgagggtccggg

SEQ ID NO: 47 - DNA, 33 bp, Homo sapiens
  hgd47 DNAzyme against GATA-3mRNA (1)..(33)
tggggtggaggctagctacaacgaagcgatggg

SEQ ID NO: 48 - DNA, 33 bp, Homo sapiens
  hgd48 DNAzyme against GATA-3mRNA (1)..(33)
cttgaggcaggctagctacaacgatctttctcg

SEQ ID NO: 49 - DNA, 33 bp, Homo sapiens
  hgd49 DNAzyme against GATA-3mRNA (1)..(33)
cacctggtaggctagctacaacgattgaggcac

SEQ ID NO: 50 - DNA, 33 bp, Homo sapiens
  hgd50 DNAzyme against GATA-3mRNA (1)..(33)
gcaggggcaggctagctacaacgactggtactt

SEQ ID NO: 51 - DNA, 33 bp, Homo sapiens
  hgd51 DNAzyme against GATA-3mRNA (1)..(33)
ccagcttcaggctagctacaacgagctgtcggg

SEQ ID NO: 52 - DNA, 33 bp, Homo sapiens
  hgd52 DNAzyme against GATA-3mRNA (1)..(33)
gtgggacgaggctagctacaacgatccagcttc

SEQ ID NO: 53 - DNA, 33 bp, Homo sapiens
  hgd53 DNAzyme against GATA-3mRNA (1)..(33)
ggagtgggaggctagctacaacgagactccagc

SEQ ID NO: 54 - DNA, 33 bp, Homo sapiens
  hgd54 DNAzyme against GATA-3mRNA (1)..(33)
atgctgccaggctagctacaacgagggagtggg

SEQ ID NO: 55 - DNA, 33 bp, Homo sapiens
  hgd55 DNAzyme against GATA-3mRNA (1)..(33)
gggcggtcaggctagctacaacgagctgccacg

SEQ ID NO: 56 - DNA, 33 bp, Homo sapiens
  hgd56 DNAzyme against GATA-3mRNA (1)..(33)
gaggctccaggctagctacaacgaccagggcgg

SEQ ID NO: 57 - DNA, 33 bp, Homo sapiens
  hgd57 DNAzyme against GATA-3mRNA (1)..(33)
gtgggtcgaggctagctacaacgagaggaggct

SEQ ID NO: 58 - DNA, 33 bp, Homo sapiens
  hgd58 DNAzyme against GATA-3mRNA (1)..(33)
aggtggtgaggctagctacaacgaggggtggtg

SEQ ID NO: 59 - DNA, 33 bp, Homo sapiens
  hgd59 DNAzyme against GATA-3mRNA (1)..(33)
actcgggcaggctagctacaacgagtagggcgg

SEQ ID NO: 60 - DNA, 33 bp, Homo sapiens
  hgd60 DNAzyme against GATA-3mRNA (1)..(33)
ggagctgtaggctagctacaacgatcgggcacg

SEQ ID NO: 61 - DNA, 33 bp, Homo sapiens
  hgd61 DNAzyme against GATA-3mRNA (1)..(33)
ggacttgcaggctagctacaacgaccgaagccg

SEQ ID NO: 62 - DNA, 33 bp, Homo sapiens
  hgd62 DNAzyme against GATA-3mRNA (1)..(33)
gggcctggaggctagctacaacgattgcatccg

SEQ ID NO: 63 - DNA, 33 bp, Homo sapiens
  hgd63 DNAzyme against GATA-3mRNA (1)..(33)
tgtgctggaggctagctacaacgacgggccttg

SEQ ID NO: 64 - DNA, 33 bp, Homo sapiens
  hgd64 DNAzyme against GATA-3mRNA (1)..(33)
gttcacacaggctagctacaacgatccctgcct

SEQ ID NO: 65 - DNA, 33 bp, Homo sapiens
  hgd65 DNAzyme against GATA-3mRNA (1)..(33)
cagttcacaggctagctacaacgaactccctgc

SEQ ID NO: 66 - DNA, 33 bp, Homo sapiens
  hgd66 DNAzyme against GATA-3mRNA (1)..(33)
cacagttcaggctagctacaacgaacactccct

SEQ ID NO: 67 - DNA, 33 bp, Homo sapiens
  hgd67 DNAzyme against GATA-3mRNA (1)..(33)
gttgccccaggctagctacaacgaagttcacac

SEQ ID NO: 68 - DNA, 33 bp, Homo sapiens
  hgd68 DNAzyme against GATA-3mRNA (1)..(33)
tcgccgccaggctagctacaacgaagtggggtc

SEQ ID NO: 69 - DNA, 33 bp, Homo sapiens
  hgd69 DNAzyme against GATA-3mRNA (1)..(33)
cccgtgccaggctagctacaacgactcgccgcc

SEQ ID NO: 70 - DNA, 33 bp, Homo sapiens
  hgd70 DNAzyme against GATA-3mRNA (1)..(33)
ggcgttgcaggctagctacaacgaaggtagtgt

SEQ ID NO: 71 - DNA, 33 bp, Homo sapiens
  td1 DNAzyme against T-bet mRNA (1)..(33)
tggcttctaggctagctacaacgagccctcgtc

SEQ ID NO: 72 - DNA, 33 bp, Homo sapiens
  td2 DNAzyme against T-bet mRNA (1)..(33)
gggctctgaggctagctacaacgagcctggctt

SEQ ID NO: 73 - DNA, 33 bp, Homo sapiens
  td3 DNAzyme against T-bet mRNA (1)..(33)
gggaccccaggctagctacaacgacggagcccg

SEQ ID NO: 74 - DNA, 33 bp, Homo sapiens
  td4 DNAzyme against T-bet mRNA (1)..(33)
ggtgggggaggctagctacaacgacccaccgga

SEQ ID NO: 75 - DNA, 33 bp, Homo sapiens
  td5 DNAzyme against T-bet mRNA (1)..(33)
ggcgggggaggctagctacaacgaccgagggcc

SEQ ID NO: 76 - DNA, 33 bp, Homo sapiens
  td6 DNAzyme against T-bet mRNA (1)..(33)
gggctgggaggctagctacaacgagggcaggga

SEQ ID NO: 77 - DNA, 33 bp, Homo sapiens
  td7 DNAzyme against T-bet mRNA (1)..(33)
cgtcgaggaggctagctacaacgaccgcccctc

SEQ ID NO: 78 - DNA, 33 bp, Homo sapiens
  td8 DNAzyme against T-bet mRNA (1)..(33)
gggctggcaggctagctacaacgacttcccgta

SEQ ID NO: 79 - DNA, 33 bp, Homo sapiens
  td9 DNAzyme against T-bet mRNA (1)..(33)
cgatgcccaggctagctacaacgaccggggcgg

SEQ ID NO: 80 - DNA, 33 bp, Homo sapiens
  td10 DNAzyme against T-bet mRNA (1)..(33)
gctccacgaggctagctacaacgagcccatccg

SEQ ID NO: 81 - DNA, 33 bp, Homo sapiens
  td11 DNAzyme against T-bet mRNA (1)..(33)
ccggctccaggctagctacaacgagatgcccat

SEQ ID NO: 82 - DNA, 33 bp, Homo sapiens
  td12 DNAzyme against T-bet mRNA (1)..(33)
tctccgcaaggctagctacaacgaccggctcca

SEQ ID NO: 83 - DNA, 33 bp, Homo sapiens
  td13 DNAzyme against T-bet mRNA (1)..(33)
ccgtcagcaggctagctacaacgagtctccgca

SEQ ID NO: 84 - DNA, 33 bp, Homo sapiens
  td14 DNAzyme against T-bet mRNA (1)..(33)
tccccggcaggctagctacaacgacggctcggt

SEQ ID NO: 85 - DNA, 33 bp, Homo sapiens
  td15 DNAzyme against T-bet mRNA (1)..(33)
cccccgcgaggctagctacaacgagctcgtccg

SEQ ID NO: 86 - DNA, 33 bp, Homo sapiens
  td16 DNAzyme against T-bet mRNA (1)..(33)
gtagggagaggctagctacaacgacccaggctg

SEQ ID NO: 87 - DNA, 33 bp, Homo sapiens
  td17 DNAzyme against T-bet mRNA (1)..(33)
gggcgggcaggctagctacaacgacaaggcgcc

SEQ ID NO: 88 - DNA, 33 bp, Homo sapiens
  td18 DNAzyme against T-bet mRNA (1)..(33)
cgggaaggaggctagctacaacgatcgcccgcg

SEQ ID NO: 89 - DNA, 33 bp, Homo sapiens
  td19 DNAzyme against T-bet mRNA (1)..(33)
tagtcctcaggctagctacaacgagcggccccg

SEQ ID NO: 90 - DNA, 33 bp, Homo sapiens
  td20 DNAzyme against T-bet mRNA (1)..(33)
tccccgacaggctagctacaacgactccagtcc

SEQ ID NO: 91 - DNA, 33 bp, Homo sapiens
  td21 DNAzyme against T-bet mRNA (1)..(33)
tttccccgaggctagctacaacgaacctccagt

SEQ ID NO: 92 - DNA, 33 bp, Homo sapiens
  td22 DNAzyme against T-bet mRNA (1)..(33)
tgagcgcgaggctagctacaacgacctcagttt

SEQ ID NO: 93 - DNA, 33 bp, Homo sapiens
  td23 DNAzyme against T-bet mRNA (1)..(33)
ggaccacaaggctagctacaacgaaggtggttg

SEQ ID NO: 94 - DNA, 33 bp, Homo sapiens
  td24 DNAzyme against T-bet mRNA (1)..(33)
cttggaccaggctagctacaacgaaacaggtgg

SEQ ID NO: 95 - DNA, 33 bp, Homo sapiens
  td25 DNAzyme against T-bet mRNA (1)..(33)
aaacttggaggctagctacaacgacacaacagg

SEQ ID NO: 96 - DNA, 33 bp, Homo sapiens
  td26 DNAzyme against T-bet mRNA (1)..(33)
ctgattaaaggctagctacaacgattggaccac

SEQ ID NO: 97 - DNA, 33 bp, Homo sapiens
  td27 DNAzyme against T-bet mRNA (1)..(33)
tggtgctgaggctagctacaacgataaacttgg

SEQ ID NO: 98 - DNA, 33 bp, Homo sapiens
  td28 DNAzyme against T-bet mRNA (1)..(33)
tgatgatcaggctagctacaacgactctgtctg

SEQ ID NO: 99 - DNA, 33 bp, Homo sapiens
  td29 DNAzyme against T-bet mRNA (1)..(33)
tggtgatgaggctagctacaacgacatctctgt

SEQ ID NO: 100 - DNA, 33 bp, Homo sapiens
  td30 DNAzyme against T-bet mRNA (1)..(33)
gcttggtgaggctagctacaacgagatcatctc

SEQ ID NO: 101 - DNA, 33 bp, Homo sapiens
  td31 DNAzyme against T-bet mRNA (1)..(33)
atgggaacaggctagctacaacgaccgccgtcc

SEQ ID NO: 102 - DNA, 33 bp, Homo sapiens
  td32 DNAzyme against T-bet mRNA (1)..(33)
gaatgggaaggctagctacaacgaatccgccgt

SEQ ID NO: 103 - DNA, 33 bp, Homo sapiens
  td33 DNAzyme against T-bet mRNA (1)..(33)
tgacaggaaggctagctacaacgagggaacatc

SEQ ID NO: 104 - DNA, 33 bp, Homo sapiens
  td34 DNAzyme against T-bet mRNA (1)..(33)
agtaaatgaggctagctacaacgaaggaatggg

SEQ ID NO: 105 - DNA, 33 bp, Homo sapiens
  td35 DNAzyme against T-bet mRNA (1)..(33)
cacagtaaaggctagctacaacgagacaggaat

SEQ ID NO: 106 - DNA, 33 bp, Homo sapiens
  td36 DNAzyme against T-bet mRNA (1)..(33)
gcccggccaggctagctacaacgaagtaaatga

SEQ ID NO: 107 - DNA, 33 bp, Homo sapiens
  td37 DNAzyme against T-bet mRNA (1)..(33)
ccacaaacaggctagctacaacgacctgtagtg

SEQ ID NO: 108 - DNA, 33 bp, Homo sapiens
  td38 DNAzyme against T-bet mRNA (1)..(33)
gtccacaaaggctagctacaacgaatcctgtag

SEQ ID NO: 109 - DNA, 33 bp, Homo sapiens
  td39 DNAzyme against T-bet mRNA (1)..(33)
ccacgtccaggctagctacaacgaaaacatcct

SEQ ID NO: 110 - DNA, 33 bp, Homo sapiens
  td40 DNAzyme against T-bet mRNA (1)..(33)
ccaagaccaggctagctacaacgagtccacaaa

SEQ ID NO: 111 - DNA, 33 bp, Homo sapiens
  td41 DNAzyme against T-bet mRNA (1)..(33)
ccaccaagaggctagctacaacgacacgtccac

SEQ ID NO: 112 - DNA, 33 bp, Homo sapiens
  td42 DNAzyme against T-bet mRNA (1)..(33)
gctggtccaggctagctacaacgacaagaccac

SEQ ID NO: 113 - DNA, 33 bp, Homo sapiens
  td43 DNAzyme against T-bet mRNA (1)..(33)
gctctggtaggctagctacaacgacgccagtgg

SEQ ID NO: 114 - DNA, 33 bp, Homo sapiens
  td44 DNAzyme against T-bet mRNA (1)..(33)
ctgcacccaggctagctacaacgattgccgctc

SEQ ID NO: 115 - DNA, 33 bp, Homo sapiens
  td45 DNAzyme against T-bet mRNA (1)..(33)
cacactgcaggctagctacaacgaccacttgcc

SEQ ID NO: 116 - DNA, 33 bp, Homo sapiens
  td46 DNAzyme against T-bet mRNA (1)..(33)
ctttccacaggctagctacaacgatgcacccac

SEQ ID NO: 117 - DNA, 33 bp, Homo sapiens
  td47 DNAzyme against T-bet mRNA (1)..(33)
gcctttccaggctagctacaacgaactgcaccc

SEQ ID NO: 118 - DNA, 33 bp, Homo sapiens
  td48 DNAzyme against T-bet mRNA (1)..(33)
ttcctggcaggctagctacaacgagctgccctc

SEQ ID NO: 119 - DNA, 33 bp, Homo sapiens
  td49 DNAzyme against T-bet mRNA (1)..(33)
gtggacgtaggctagctacaacgaaggcggttt

SEQ ID NO: 120 - DNA, 33 bp, Homo sapiens
  td50 DNAzyme against T-bet mRNA (1)..(33)
ccgggtggaggctagctacaacgagtacaggcg

SEQ ID NO: 121 - DNA, 33 bp, Homo sapiens
  td51 DNAzyme against T-bet mRNA (1)..(33)
cctggcgcaggctagctacaacgaccagtgcgc

SEQ ID NO: 122 - DNA, 33 bp, Homo sapiens
  td52 DNAzyme against T-bet mRNA (1)..(33)
caaatgaaaggctagctacaacgattcctggcg

SEQ ID NO: 123 - DNA, 33 bp, Homo sapiens
  td53 DNAzyme against T-bet mRNA (1)..(33)
tttcccaaaggctagctacaacgagaaacttcc

SEQ ID NO: 124 - DNA, 33 bp, Homo sapiens
  td54 DNAzyme against T-bet mRNA (1)..(33)
attgttggaggctagctacaacgagcccccttg

SEQ ID NO: 125 - DNA, 33 bp, Homo sapiens
  td55 DNAzyme against T-bet mRNA (1)..(33)
tgggtcacaggctagctacaacgatgttggacg

SEQ ID NO: 126 - DNA, 33 bp, Homo sapiens
  td56 DNAzyme against T-bet mRNA (1)..(33)
tctgggtcaggctagctacaacgaattgttgga

SEQ ID NO: 127 - DNA, 33 bp, Homo sapiens
  td57 DNAzyme against T-bet mRNA (1)..(33)
gcacaatcaggctagctacaacgactgggtcac

SEQ ID NO: 128 - DNA, 33 bp, Homo sapiens
  td58 DNAzyme against T-bet mRNA (1)..(33)
ggagcacaaggctagctacaacgacatctgggt

SEQ ID NO: 129 - DNA, 33 bp, Homo sapiens
  td59 DNAzyme against T-bet mRNA (1)..(33)
actggagcaggctagctacaacgaaatcatctg

SEQ ID NO: 130 - DNA, 33 bp, Homo sapiens
  td60 DNAzyme against T-bet mRNA (1)..(33)
atggagggaggctagctacaacgatggagcaca

SEQ ID NO: 131 - DNA, 33 bp, Homo sapiens
  td61 DNAzyme against T-bet mRNA (1)..(33)
tggtacttaggctagctacaacgaggagggact

SEQ ID NO: 132 - DNA, 33 bp, Homo sapiens
  td62 DNAzyme against T-bet mRNA (1)..(33)
gggctggtaggctagctacaacgattatggagg

SEQ ID NO: 133 - DNA, 33 bp, Homo sapiens
  td63 DNAzyme against T-bet mRNA (1)..(33)
tcaacgataggctagctacaacgagcagccggg

SEQ ID NO: 134 - DNA, 33 bp, Homo sapiens
  td64 DNAzyme against T-bet mRNA (1)..(33)
cctcaacgaggctagctacaacgaatgcagccg

SEQ ID NO: 135 - DNA, 33 bp, Homo sapiens
  td65 DNAzyme against T-bet mRNA (1)..(33)
tcacctcaaggctagctacaacgagatatgcag

SEQ ID NO: 136 - DNA, 33 bp, Homo sapiens
  td66 DNAzyme against T-bet mRNA (1)..(33)
cgtcgttcaggctagctacaacgactcaacgat

SEQ ID NO: 137 - DNA, 33 bp, Homo sapiens
  td67 DNAzyme against T-bet mRNA (1)..(33)
gtaaagataggctagctacaacgagcgtgttgg

SEQ ID NO: 138 - DNA, 33 bp, Homo sapiens
  td68 DNAzyme against T-bet mRNA (1)..(33)
aagtaaagaggctagctacaacgaatgcgtgtt

SEQ ID NO: 139 - DNA, 33 bp, Homo sapiens
  td69 DNAzyme against T-bet mRNA (1)..(33)
ggcaatgaaggctagctacaacgatgggtttct

SEQ ID NO: 140 - DNA, 33 bp, Homo sapiens
  td70 DNAzyme against T-bet mRNA (1)..(33)
tcacggcaaggctagctacaacgagaactgggt

SEQ ID NO: 141 - DNA, 33 bp, Homo sapiens
  td71 DNAzyme against T-bet mRNA (1)..(33)
aggcagtcaggctagctacaacgaggcaatgaa

SEQ ID NO: 142 - DNA, 33 bp, Homo sapiens
  td72 DNAzyme against T-bet mRNA (1)..(33)
atctcggcaggctagctacaacgatctggtagg

SEQ ID NO: 143 - DNA, 33 bp, Homo sapiens
  td73 DNAzyme against T-bet mRNA (1)..(33)
gctgagtaaggctagctacaacgactcggcatt

SEQ ID NO: 144 - DNA, 33 bp, Homo sapiens
  td74 DNAzyme against T-bet mRNA (1)..(33)
tattatcaaggctagctacaacgatttcagctg

SEQ ID NO: 145 - DNA, 33 bp, Homo sapiens
  td75 DNAzyme against T-bet mRNA (1)..(33)
gggttattaggctagctacaacgacaattttca

SEQ ID NO: 146 - DNA, 33 bp, Homo sapiens
  td76 DNAzyme against T-bet mRNA (1)..(33)
aaggggttaggctagctacaacgatatcaattt

SEQ ID NO: 147 - DNA, 33 bp, Homo sapiens
  td77 DNAzyme against T-bet mRNA (1)..(33)
ctcccggaaggctagctacaacgacctttggca

SEQ ID NO: 148 - DNA, 33 bp, Homo sapiens
  td78 DNAzyme against T-bet mRNA (1)..(33)
gtacatggaggctagctacaacgatcaaagttc